European Patent Application EP 4 574 971 A2, published June 25, 2025. Title: PROTEOMIC SCREENING FOR LYSOSOMAL STORAGE DISEASES. Applicant: Seattle Children's Hospital d/b/a Seattle Children's Research Institute. The sequence listing filed with the application follows.

SEQUENCE LISTING (87 sequences)

SEQ ID NO: 1 - protein, 13 aa, Homo sapiens
LGGPGDSFHTPPR

SEQ ID NO: 2 - protein, 13 aa, Homo sapiens
GVPPGPGLVYVTR

SEQ ID NO: 3 - protein, 8 aa, Homo sapiens
TTPTFFPK

SEQ ID NO: 4 - protein, 17 aa, Homo sapiens
STGGILDVYIFLGPEPK

SEQ ID NO: 5 - protein, 10 aa, Homo sapiens
WGYSSTAITR

SEQ ID NO: 6 - protein, 8 aa, Homo sapiens
STFAGHGR

SEQ ID NO: 7 - protein, 16 aa, Homo sapiens
GELFWDDGESLEVLER

SEQ ID NO: 8 - protein, 10 aa, Homo sapiens
NNTIVNELVR

SEQ ID NO: 9 - protein, 12 aa, Homo sapiens
VTSEGAGLQLQK

SEQ ID NO: 10 - protein, 5 aa, synthetic construct
  source 1..5: note = anti-IDUA 218 VH CDR1
RYWMH

SEQ ID NO: 11 - protein, 17 aa, synthetic construct
  source 1..17: note = anti-IDUA 218 VH CDR2
EINPSNGGTNYNEKFKN

SEQ ID NO: 12 - protein, 4 aa, synthetic construct
  source 1..4: note = anti-IDUA 218 VH CDR3
AMDY

SEQ ID NO: 13 - protein, 16 aa, synthetic construct
  source 1..16: note = anti-IDUA 218 VL CDR1
KSSQSLLHSDGKTYLN

SEQ ID NO: 14 - protein, 7 aa, synthetic construct
  source 1..7: note = anti-IDUA 218 VL CDR2
LVSKLDS

SEQ ID NO: 15 - protein, 9 aa, synthetic construct
  source 1..9: note = anti-IDUA 218 VL CDR3
WQGLHFPWT

SEQ ID NO: 16 - DNA, 396 bp, synthetic construct
  source 1..396: mol_type = other DNA; note = anti-IDUA 218 variable heavy domain coding sequence with leader sequence
atgggatggagctatatcatcctctttttggtagcaacagttacagatgtccactcccaggtccaactgcagcagcctgggactgagcttgtgaagcctggggcttcagtgaagttgtcctgcaaggcttctggctacaccttcaccaggtactggatgcactgggtgaagcagaggcctggacaaggccttgagtggattggagagattaatcctagcaatggtgggactaactacaatgagaagttcaagaacaaggccacactgaatgttgacaaatcctccagcacagcctacatgcaactcagcagcctgacatctgaggactctgcggtctattactgtacgttagctatggactactggggtcaaggaacctcagtcaccgtctcctca

SEQ ID NO: 17 - protein, 132 aa, synthetic construct
  source 1..132: note = anti-IDUA 218 variable heavy domain amino acid sequence with leader sequence
MGWSYIILFLVATVTDVHSQVQLQQPGTELVKPGASVKLSCKASGYTFTRYWMHWVKQRPGQGLEWIGEINPSNGGTNYNEKFKNKATLNVDKSSSTAYMQLSSLTSEDSAVYYCTLAMDYWGQGTSVTVSS

SEQ ID NO: 18 - protein, 113 aa, synthetic construct
  source 1..113: note = anti-IDUA 218 variable heavy domain amino acid sequence without leader sequence
QVQLQQPGTELVKPGASVKLSCKASGYTFTRYWMHWVKQRPGQGLEWIGEINPSNGGTNYNEKFKNKATLNVDKSSSTAYMQLSSLTSEDSAVYYCTLAMDYWGQGTSVTVSS

SEQ ID NO: 19 - DNA, 393 bp, synthetic construct
  source 1..393: mol_type = other DNA; note = anti-IDUA 218 variable light domain coding sequence with leader sequence
atgagtcctgcccagttcctgtttctgttagtgctctggattcgggaaaccaacggtgatgttgtgatgacccagactccactcactttgtcggttaccattggacaaccagcctccatctcttgcaagtcaagtcagagcctcttacatagtgatggaaagacatatttgaattggtcgttacagaggccaggccagtctccaaagcgcctaatctatctggtgtctaaactggactctggagtccctgacaggttcactggcagtggatcagggacagatttcacactgaaaatcagcagagtggaggctgaggatttgggagtttattattgctggcaaggtttacattttccgtggacgttcggtggaggcaccaagctggaaatcaaa

SEQ ID NO: 20 - protein, 131 aa, synthetic construct
  source 1..131: note = anti-IDUA 218 variable light domain amino acid sequence with leader sequence
MSPAQFLFLLVLWIRETNGDVVMTQTPLTLSVTIGQPASISCKSSQSLLHSDGKTYLNWSLQRPGQSPKRLIYLVSKLDSGVPDRFTGSGSGTDFTLKISRVEAEDLGVYYCWQGLHFPWTFGGGTKLEIK

SEQ ID NO: 21 - protein, 112 aa, synthetic construct
  source 1..112: note = anti-IDUA 218 variable light domain amino acid sequence without leader sequence
DVVMTQTPLTLSVTIGQPASISCKSSQSLLHSDGKTYLNWSLQRPGQSPKRLIYLVSKLDSGVPDRFTGSGSGTDFTLKISRVEAEDLGVYYCWQGLHFPWTFGGGTKLEIK

SEQ ID NO: 22 - protein, 5 aa, synthetic construct
  source 1..5: note = anti-IDUA 462 VH CDR1
DTYMH

SEQ ID NO: 23 - protein, 17 aa, synthetic construct
  source 1..17: note = anti-IDUA 462 VH CDR2
RIDPANGNTKYGPKFQG

SEQ ID NO: 24 - protein, 8 aa, synthetic construct
  source 1..8: note = anti-IDUA 462 VH CDR3
TARAPFAY

SEQ ID NO: 25 - protein, 16 aa, synthetic construct
  source 1..16: note = anti-IDUA 462 VL CDR1
RSSKSLLYKDGKTYLN

SEQ ID NO: 26 - protein, 7 aa, synthetic construct
  source 1..7: note = anti-IDUA 462 VL CDR2
WMSTRAS

SEQ ID NO: 27 - protein, 9 aa, synthetic construct
  source 1..9: note = anti-IDUA 462 VL CDR3
QQVVEYPFT

SEQ ID NO: 28 - DNA, 408 bp, synthetic construct
  source 1..408: mol_type = other DNA; note = anti-IDUA 462 variable heavy domain coding sequence with leader sequence
atgaaatgcagctgggttatcttcttcctgatggcagtggttacaggggtcaattcagaggttcagctgcagcagtctggggcagagcttgtgaagccaggggcctcagtcaagttgtcctgcacagcttctggcttcaacattaaagacacctatatgcactgggtgaaccagaggcctgaacagggcctggagtggattggaaggattgatcctgcgaatggtaatactaaatatggcccgaagttccagggcaaggccactataacagcagacacatcctccaacacagcctacctgcagctcagcagcctgacatctgaggacactgccgtctattactgtgcccagacagctcgggccccgtttgcttactggggccaagggactctggtcactgtctctgca

SEQ ID NO: 29 - protein, 136 aa, synthetic construct
  source 1..136: note = anti-IDUA 462 variable heavy domain amino acid sequence with leader sequence
MKCSWVIFFLMAVVTGVNSEVQLQQSGAELVKPGASVKLSCTASGFNIKDTYMHWVNQRPEQGLEWIGRIDPANGNTKYGPKFQGKATITADTSSNTAYLQLSSLTSEDTAVYYCAQTARAPFAYWGQGTLVTVSA

SEQ ID NO: 30 - protein, 117 aa, synthetic construct
  source 1..117: note = anti-IDUA 462 variable heavy domain amino acid sequence without leader sequence
EVQLQQSGAELVKPGASVKLSCTASGFNIKDTYMHWVNQRPEQGLEWIGRIDPANGNTKYGPKFQGKATITADTSSNTAYLQLSSLTSEDTAVYYCAQTARAPFAYWGQGTLVTVSA

SEQ ID NO: 31 - DNA, 396 bp, synthetic construct
  source 1..396: mol_type = other DNA; note = anti-IDUA 462 variable light domain coding sequence with leader sequence
atgaggtgctctcttcagttcttggggatgcttatgttctggatctctggagtcagtggggatattgtgataacccaggatgaagtctccaatcctgtcacttctggagaatcagtttccatctcctgcaggtctagtaagagtctcctatataaggatgggaagacatacttgaattggtttctgcagaggccaggacagtctcctcagctcctggtctattggatgtccacccgtgcatcaggagtctcagaccggtttagtggcagtgggtcaggaacagatttcacactgaaaatcagtagagtgaaggctgaggatgtcggtatgtattactgtcaacaagttgtagagtatccattcacgttcggcacggggacaaaattggaaataaaa

SEQ ID NO: 32 - protein, 132 aa, synthetic construct
  source 1..132: note = anti-IDUA 462 variable light domain amino acid sequence with leader sequence
MRCSLQFLGMLMFWISGVSGDIVITQDEVSNPVTSGESVSISCRSSKSLLYKDGKTYLNWFLQRPGQSPQLLVYWMSTRASGVSDRFSGSGSGTDFTLKISRVKAEDVGMYYCQQVVEYPFTFGTGTKLEIK

SEQ ID NO: 33 - protein, 112 aa, synthetic construct
  source 1..112: note = anti-IDUA 462 variable light domain amino acid sequence without leader sequence
DIVITQDEVSNPVTSGESVSISCRSSKSLLYKDGKTYLNWFLQRPGQSPQLLVYWMSTRASGVSDRFSGSGSGTDFTLKISRVKAEDVGMYYCQQVVEYPFTFGTGTKLEIK

SEQ ID NO: 34 - protein, 11 aa, synthetic construct
  source 1..11: note = Gly-Ser linker
GGSGGGSGGSG

SEQ ID NO: 35 - protein, 10 aa, synthetic construct
  source 1..10: note = Gly-Ser linker
GGSGGGSGSG

SEQ ID NO: 36 - protein, 8 aa, synthetic construct
  source 1..8: note = Gly-Ser linker
GGSGGGSG

SEQ ID NO: 37 - protein, 10 aa, synthetic construct
  source 1..10: note = Gly-Ser linker
GGGGSGGGGS

SEQ ID NO: 38 - protein, 8 aa, synthetic construct
  source 1..8: note = Gly-Ser linker
GGGSGGGS

SEQ ID NO: 39 - protein, 6 aa, synthetic construct
  source 1..6: note = Gly-Ser linker
GGSGGS

SEQ ID NO: 40 - DNA, 339 bp, synthetic construct
  source 1..339: mol_type = other DNA; note = anti-IDUA 218 variable heavy domain coding sequence without leader sequence
caggtccaactgcagcagcctgggactgagcttgtgaagcctggggcttcagtgaagttgtcctgcaaggcttctggctacaccttcaccaggtactggatgcactgggtgaagcagaggcctggacaaggccttgagtggattggagagattaatcctagcaatggtgggactaactacaatgagaagttcaagaacaaggccacactgaatgttgacaaatcctccagcacagcctacatgcaactcagcagcctgacatctgaggactctgcggtctattactgtacgttagctatggactactggggtcaaggaacctcagtcaccgtctcctca

SEQ ID NO: 41 - DNA, 336 bp, synthetic construct
  source 1..336: mol_type = other DNA; note = anti-IDUA 218 variable light domain coding sequence without leader sequence
gatgttgtgatgacccagactccactcactttgtcggttaccattggacaaccagcctccatctcttgcaagtcaagtcagagcctcttacatagtgatggaaagacatatttgaattggtcgttacagaggccaggccagtctccaaagcgcctaatctatctggtgtctaaactggactctggagtccctgacaggttcactggcagtggatcagggacagatttcacactgaaaatcagcagagtggaggctgaggatttgggagtttattattgctggcaaggtttacattttccgtggacgttcggtggaggcaccaagctggaaatcaaa

SEQ ID NO: 42 - DNA, 351 bp, synthetic construct
  source 1..351: mol_type = other DNA; note = anti-IDUA 462 variable heavy domain coding sequence without leader sequence
gaggttcagctgcagcagtctggggcagagcttgtgaagccaggggcctcagtcaagttgtcctgcacagcttctggcttcaacattaaagacacctatatgcactgggtgaaccagaggcctgaacagggcctggagtggattggaaggattgatcctgcgaatggtaatactaaatatggcccgaagttccagggcaaggccactataacagcagacacatcctccaacacagcctacctgcagctcagcagcctgacatctgaggacactgccgtctattactgtgcccagacagctcgggccccgtttgcttactggggccaagggactctggtcactgtctctgca

SEQ ID NO: 43 - DNA, 336 bp, synthetic construct
  source 1..336: mol_type = other DNA; note = anti-IDUA 462 variable light domain coding sequence without leader sequence
gatattgtgataacccaggatgaagtctccaatcctgtcacttctggagaatcagtttccatctcctgcaggtctagtaagagtctcctatataaggatgggaagacatacttgaattggtttctgcagaggccaggacagtctcctcagctcctggtctattggatgtccacccgtgcatcaggagtctcagaccggtttagtggcagtgggtcaggaacagatttcacactgaaaatcagtagagtgaaggctgaggatgtcggtatgtattactgtcaacaagttgtagagtatccattcacgttcggcacggggacaaaattggaaataaaa

SEQ ID NO: 44 - protein, 5 aa, synthetic construct
  source 1..5: note = anti-GAA 155 VH CDR1
SYVMS

SEQ ID NO: 45 - protein, 16 aa, synthetic construct
  source 1..16: note = anti-GAA 155 VH CDR2
VISTGGITYYANWAKG

SEQ ID NO: 46 - protein, 8 aa, synthetic construct
  source 1..8: note = anti-GAA 155 VH CDR3
GFSGDNYV

SEQ ID NO: 47 - protein, 13 aa, synthetic construct
  source 1..13: note = anti-GAA 155 VL CDR1
QSSQNVHSNNYLS

SEQ ID NO: 48 - protein, 7 aa, synthetic construct
  source 1..7: note = anti-GAA 155 VL CDR2
LASTLAS

SEQ ID NO: 49 - protein, 10 aa, synthetic construct
  source 1..10: note = anti-GAA 155 VL CDR3
AGDYTTNIYV

SEQ ID NO: 50 - DNA, 1368 bp, synthetic construct
  source 1..1368: mol_type = other DNA; note = anti-GAA 155 (clone pEB0613A-3B2-H1) heavy chain coding sequence with leader sequence
atggagactgggctgcgctggcttctcctggtcgctgtgctcaaaggtgtccagtgtcagtcggtggaggagtccgggggtcgcctggtcacgcctgggacacccctgacactcacctgcacagcctctggattctccctcaatagttatgtaatgagttgggtccgccaggctccaggggaggggctggaatggatcggggtcattagtactggtggtatcacatactacgcgaactgggcaaaaggccgattcaccatctccaaaacctcgaccacggtggatctgaaaatcaccagtccgagaaccgaggacacggccacctatttctgtgccagaggatttagtggtgataattacgtctggggcccaggcaccctggtcaccgtctccttcgggcaacctaaggctccatcagtcttcccactggccccctgctgcggggacacacccagctccacggtgaccctgggctgcctggtcaaaggctacctcccggagccagtgaccgtgacctggaactcgggcaccctcaccaatggggtacgcaccttcccgtccgtccggcagtcctcaggcctctactcgctgagcagcgtggtgagcgtgacctcaagcagccagcccgtcacctgcaacgtggcccacccagccaccaacaccaaagtggacaagaccgttgcgccctcgacatgcagcaagcccatgtgcccaccccctgaactcctggggggaccgtctgtcttcatcttccccccaaaacccaaggacaccctcatgatctcacgcacccccgaggtcacatgcgtggtggtggacgtgagccaggatgaccccgaggtgcagttcacatggtacataaacaacgagcaggtgcgcaccgcccggccgccgctacgggagcagcagttcaacagcacgatccgcgtggtcagcaccctccccatcgcgcaccaggactggctgaggggcaaggagttcaagtgcaaagtccacaacaaggcactcccggcccccatcgagaaaaccatctccaaagccagagggcagcccctggagccgaaggtctacaccatgggccctccccgggaggagctgagcagcaggtcggtcagcctgacctgcatgatcaacggcttctacccttccgacatctcggtggagtgggagaagaacgggaaggcagaggacaactacaagaccacgccggccgtgctggacagcgacggctcctacttcctctacagcaagctctcagtgcccacgagtgagtggcagcggggcgacgtcttcacctgctccgtgatgcacgaggccttgcacaaccactacacgcagaagtccatctcccgctctccgggtaaatga

SEQ ID NO: 51 - DNA, 1311 bp, synthetic construct
  source 1..1311: mol_type = other DNA; note = anti-GAA 155 (clone pEB0613A-3B2-H1) heavy chain coding sequence without leader sequence
cagtcggtggaggagtccgggggtcgcctggtcacgcctgggacacccctgacactcacctgcacagcctctggattctccctcaatagttatgtaatgagttgggtccgccaggctccaggggaggggctggaatggatcggggtcattagtactggtggtatcacatactacgcgaactgggcaaaaggccgattcaccatctccaaaacctcgaccacggtggatctgaaaatcaccagtccgagaaccgaggacacggccacctatttctgtgccagaggatttagtggtgataattacgtctggggcccaggcaccctggtcaccgtctccttcgggcaacctaaggctccatcagtcttcccactggccccctgctgcggggacacacccagctccacggtgaccctgggctgcctggtcaaaggctacctcccggagccagtgaccgtgacctggaactcgggcaccctcaccaatggggtacgcaccttcccgtccgtccggcagtcctcaggcctctactcgctgagcagcgtggtgagcgtgacctcaagcagccagcccgtcacctgcaacgtggcccacccagccaccaacaccaaagtggacaagaccgttgcgccctcgacatgcagcaagcccatgtgcccaccccctgaactcctggggggaccgtctgtcttcatcttccccccaaaacccaaggacaccctcatgatctcacgcacccccgaggtcacatgcgtggtggtggacgtgagccaggatgaccccgaggtgcagttcacatggtacataaacaacgagcaggtgcgcaccgcccggccgccgctacgggagcagcagttcaacagcacgatccgcgtggtcagcaccctccccatcgcgcaccaggactggctgaggggcaaggagttcaagtgcaaagtccacaacaaggcactcccggcccccatcgagaaaaccatctccaaagccagagggcagcccctggagccgaaggtctacaccatgggccctccccgggaggagctgagcagcaggtcggtcagcctgacctgcatgatcaacggcttctacccttccgacatctcggtggagtgggagaagaacgggaaggcagaggacaactacaagaccacgccggccgtgctggacagcgacggctcctacttcctctacagcaagctctcagtgcccacgagtgagtggcagcggggcgacgtcttcacctgctccgtgatgcacgaggccttgcacaaccactacacgcagaagtccatctcccgctctccgggtaaatga

SEQ ID NO: 52 - DNA, 396 bp, synthetic construct
  source 1..396: mol_type = other DNA; note = anti-GAA 155 (clone pEB0613A-3B2-H1) variable heavy domain coding sequence with leader sequence
atggagactgggctgcgctggcttctcctggtcgctgtgctcaaaggtgtccagtgtcagtcggtggaggagtccgggggtcgcctggtcacgcctgggacacccctgacactcacctgcacagcctctggattctccctcaatagttatgtaatgagttgggtccgccaggctccaggggaggggctggaatggatcggggtcattagtactggtggtatcacatactacgcgaactgggcaaaaggccgattcaccatctccaaaacctcgaccacggtggatctgaaaatcaccagtccgagaaccgaggacacggccacctatttctgtgccagaggatttagtggtgataattacgtctggggcccaggcaccctggtcaccgtctccttc

SEQ ID NO: 53 - DNA, 339 bp, synthetic construct
  source 1..339: mol_type = other DNA; note = anti-GAA 155 (clone pEB0613A-3B2-H1) variable heavy domain coding sequence without leader sequence
cagtcggtggaggagtccgggggtcgcctggtcacgcctgggacacccctgacactcacctgcacagcctctggattctccctcaatagttatgtaatgagttgggtccgccaggctccaggggaggggctggaatggatcggggtcattagtactggtggtatcacatactacgcgaactgggcaaaaggccgattcaccatctccaaaacctcgaccacggtggatctgaaaatcaccagtccgagaaccgaggacacggccacctatttctgtgccagaggatttagtggtgataattacgtctggggcccaggcaccctggtcaccgtctccttc

SEQ ID NO: 54 - protein, 455 aa, synthetic construct
  source 1..455: note = anti-GAA 155 heavy chain amino acid sequence with leader sequence
METGLRWLLLVAVLKGVQCQSVEESGGRLVTPGTPLTLTCTASGFSLNSYVMSWVRQAPGEGLEWIGVISTGGITYYANWAKGRFTISKTSTTVDLKITSPRTEDTATYFCARGFSGDNYVWGPGTLVTVSFGQPKAPSVFPLAPCCGDTPSSTVTLGCLVKGYLPEPVTVTWNSGTLTNGVRTFPSVRQSSGLYSLSSVVSVTSSSQPVTCNVAHPATNTKVDKTVAPSTCSKPMCPPPELLGGPSVFIFPPKPKDTLMISRTPEVTCVVVDVSQDDPEVQFTWYINNEQVRTARPPLREQQFNSTIRVVSTLPIAHQDWLRGKEFKCKVHNKALPAPIEKTISKARGQPLEPKVYTMGPPREELSSRSVSLTCMINGFYPSDISVEWEKNGKAEDNYKTTPAVLDSDGSYFLYSKLSVPTSEWQRGDVFTCSVMHEALHNHYTQKSISRSPGK

SEQ ID NO: 55 - protein, 436 aa, synthetic construct
  source 1..436: note = anti-GAA 155 heavy chain amino acid sequence without leader sequence
QSVEESGGRLVTPGTPLTLTCTASGFSLNSYVMSWVRQAPGEGLEWIGVISTGGITYYANWAKGRFTISKTSTTVDLKITSPRTEDTATYFCARGFSGDNYVWGPGTLVTVSFGQPKAPSVFPLAPCCGDTPSSTVTLGCLVKGYLPEPVTVTWNSGTLTNGVRTFPSVRQSSGLYSLSSVVSVTSSSQPVTCNVAHPATNTKVDKTVAPSTCSKPMCPPPELLGGPSVFIFPPKPKDTLMISRTPEVTCVVVDVSQDDPEVQFTWYINNEQVRTARPPLREQQFNSTIRVVSTLPIAHQDWLRGKEFKCKVHNKALPAPIEKTISKARGQPLEPKVYTMGPPREELSSRSVSLTCMINGFYPSDISVEWEKNGKAEDNYKTTPAVLDSDGSYFLYSKLSVPTSEWQRGDVFTCSVMHEALHNHYTQKSISRSPGK

SEQ ID NO: 56 - protein, 132 aa, synthetic construct
  source 1..132: note = anti-GAA 155 variable heavy domain amino acid sequence with leader sequence
METGLRWLLLVAVLKGVQCQSVEESGGRLVTPGTPLTLTCTASGFSLNSYVMSWVRQAPGEGLEWIGVISTGGITYYANWAKGRFTISKTSTTVDLKITSPRTEDTATYFCARGFSGDNYVWGPGTLVTVSF

SEQ ID NO: 57 - protein, 113 aa, synthetic construct
  source 1..113: note = anti-GAA 155 variable heavy domain amino acid sequence without leader sequence
QSVEESGGRLVTPGTPLTLTCTASGFSLNSYVMSWVRQAPGEGLEWIGVISTGGITYYANWAKGRFTISKTSTTVDLKITSPRTEDTATYFCARGFSGDNYVWGPGTLVTVSF

SEQ ID NO: 58 - DNA, 714 bp, synthetic construct
  source 1..714: mol_type = other DNA; note = anti-GAA 155 (clone pEB0613A-3B2-K3) light chain coding sequence with leader sequence
atggacacgagggcccccactcagctgctggggctcctactgctctggctcccaggtgccagatgtgctgacattgtgatgacccagactccatcttccacgtctgcggctgtgggaggcacagtcaccatcaactgccagtccagtcagaatgttcatagtaacaactacttatcctggtttcagcagaaaccagggcagcctcccaagctcctgatctatctggcttccactctggcatctggggtcccatcgcggttcaaaggcagtggctctgggacagagttcactctcaccatcagcgacctggagtgtgatgatgctgccacttactactgtgcaggcgattatactactaatatttatgttttcggcggagggaccgaggtggtggtcaaaggtgatccagttgcacctactgtcctcatcttcccaccagctgctgatcaggtggcaactggaacagtcaccatcgtgtgtgtggcgaataaatactttcccgatgtcaccgtcacctgggaggtggatggcaccacccaaacaactggcatcgagaacagtaaaacaccgcagaattctgcagattgtacctacaacctcagcagcactctgacactgaccagcacacagtacaacagccacaaagagtacacctgcaaggtgacccagggcacgacctcagtcgtccagagcttcaataggggtgactgttag

SEQ ID NO: 59 - DNA, 648 bp, synthetic construct
  source 1..648: mol_type = other DNA; note = anti-GAA 155 (clone pEB0613A-3B2-K3) light chain coding sequence without leader sequence
gctgacattgtgatgacccagactccatcttccacgtctgcggctgtgggaggcacagtcaccatcaactgccagtccagtcagaatgttcatagtaacaactacttatcctggtttcagcagaaaccagggcagcctcccaagctcctgatctatctggcttccactctggcatctggggtcccatcgcggttcaaaggcagtggctctgggacagagttcactctcaccatcagcgacctggagtgtgatgatgctgccacttactactgtgcaggcgattatactactaatatttatgttttcggcggagggaccgaggtggtggtcaaaggtgatccagttgcacctactgtcctcatcttcccaccagctgctgatcaggtggcaactggaacagtcaccatcgtgtgtgtggcgaataaatactttcccgatgtcaccgtcacctgggaggtggatggcaccacccaaacaactggcatcgagaacagtaaaacaccgcagaattctgcagattgtacctacaacctcagcagcactctgacactgaccagcacacagtacaacagccacaaagagtacacctgcaaggtgacccagggcacgacctcagtcgtccagagcttcaataggggtgactgttag

SEQ ID NO: 60 - DNA, 399 bp, synthetic construct
  source 1..399: mol_type = other DNA; note = anti-GAA 155 (clone pEB0613A-3B2-K3) variable light domain coding sequence with leader sequence
atggacacgagggcccccactcagctgctggggctcctactgctctggctcccaggtgccagatgtgctgacattgtgatgacccagactccatcttccacgtctgcggctgtgggaggcacagtcaccatcaactgccagtccagtcagaatgttcatagtaacaactacttatcctggtttcagcagaaaccagggcagcctcccaagctcctgatctatctggcttccactctggcatctggggtcccatcgcggttcaaaggcagtggctctgggacagagttcactctcaccatcagcgacctggagtgtgatgatgctgccacttactactgtgcaggcgattatactactaatatttatgttttcggcggagggaccgaggtggtggtcaaa

SEQ ID NO: 61 - DNA, 333 bp, synthetic construct
  source 1..333: mol_type = other DNA; note = anti-GAA 155 (clone pEB0613A-3B2-K3) variable light domain coding sequence without leader sequence
gctgacattgtgatgacccagactccatcttccacgtctgcggctgtgggaggcacagtcaccatcaactgccagtccagtcagaatgttcatagtaacaactacttatcctggtttcagcagaaaccagggcagcctcccaagctcctgatctatctggcttccactctggcatctggggtcccatcgcggttcaaaggcagtggctctgggacagagttcactctcaccatcagcgacctggagtgtgatgatgctgccacttactactgtgcaggcgattatactactaatatttatgttttcggcggagggaccgaggtggtggtcaaa

SEQ ID NO: 62 - protein, 237 aa, synthetic construct
  source 1..237: note = anti-GAA 155 light chain amino acid sequence with leader sequence
MDTRAPTQLLGLLLLWLPGARCADIVMTQTPSSTSAAVGGTVTINCQSSQNVHSNNYLSWFQQKPGQPPKLLIYLASTLASGVPSRFKGSGSGTEFTLTISDLECDDAATYYCAGDYTTNIYVFGGGTEVVVKGDPVAPTVLIFPPAADQVATGTVTIVCVANKYFPDVTVTWEVDGTTQTTGIENSKTPQNSADCTYNLSSTLTLTSTQYNSHKEYTCKVTQGTTSVVQSFNRGDC

SEQ ID NO: 63 - protein, 215 aa, synthetic construct
  source 1..215: note = anti-GAA 155 light chain amino acid sequence without leader sequence
ADIVMTQTPSSTSAAVGGTVTINCQSSQNVHSNNYLSWFQQKPGQPPKLLIYLASTLASGVPSRFKGSGSGTEFTLTISDLECDDAATYYCAGDYTTNIYVFGGGTEVVVKGDPVAPTVLIFPPAADQVATGTVTIVCVANKYFPDVTVTWEVDGTTQTTGIENSKTPQNSADCTYNLSSTLTLTSTQYNSHKEYTCKVTQGTTSVVQSFNRGDC

SEQ ID NO: 64 - protein, 133 aa, synthetic construct
  source 1..133: note = anti-GAA 155 variable light domain amino acid sequence with leader sequence
MDTRAPTQLLGLLLLWLPGARCADIVMTQTPSSTSAAVGGTVTINCQSSQNVHSNNYLSWFQQKPGQPPKLLIYLASTLASGVPSRFKGSGSGTEFTLTISDLECDDAATYYCAGDYTTNIYVFGGGTEVVVK

SEQ ID NO: 65 - protein, 111 aa, synthetic construct
  source 1..111: note = anti-GAA 155 variable light domain amino acid sequence without leader sequence
ADIVMTQTPSSTSAAVGGTVTINCQSSQNVHSNNYLSWFQQKPGQPPKLLIYLASTLASGVPSRFKGSGSGTEFTLTISDLECDDAATYYCAGDYTTNIYVFGGGTEVVVK

SEQ ID NO: 66 - protein, 5 aa, synthetic construct
  source 1..5: note = anti-GAA 376 VH CDR1
SVDMS

SEQ ID NO: 67 - protein, 16 aa, synthetic construct
  source 1..16: note = anti-GAA 376 VH CDR2
FSNAYHRTYYASWSKS

SEQ ID NO: 68 - protein, 11 aa, synthetic construct
  source 1..11: note = anti-GAA 376 VH CDR3
GVPGYVTKSSL

SEQ ID NO: 69 - protein, 13 aa, synthetic construct
  source 1..13: note = anti-GAA 376 VL CDR1
QASQSVYGNNELS

SEQ ID NO: 70 - protein, 7 aa, synthetic construct
  source 1..7: note = anti-GAA 376 VL CDR2
KASTLAS

SEQ ID NO: 71 - protein, 12 aa, synthetic construct
  source 1..12: note = anti-GAA 376 VL CDR3
AGYSSGVIDVSA

SEQ ID NO: 72 - DNA, 1386 bp, synthetic construct
  source 1..1386: mol_type = other DNA; note = anti-GAA 376 (clone pEB0613B-4B1-H2) heavy chain coding sequence with leader sequence
atggagactgggctgcgctggcttctcctggtcgctgtgctcaaaggtgtccagtgtcaggagcacctggtggagtccgggggaggcctggtcaaccctggaggatccctgacactcacctgcacagcctctggattctccctcaacagcgtcgacatgagctgggtccgccaggctccagggaaggggctggagtggatcggattcagtaatgcttatcataggacatactacgcgagctggtcgaaaagccgatccaccatcaccagaaacaccaacgagaacacggtgactctgaaaatgaccagtctgacagccgcggacacggccacctatttctgtgcgagaggtgttcctggttatgttactaaaagtagtctctggggcccaggcaccctggtcaccgtctcctcagggcaacctaaggctccatcagtcttcccactggccccctgctgcggggacacacccagctccacggtgaccctgggctgcctggtcaaaggctacctcccggagccagtgaccgtgacctggaactcgggcaccctcaccaatggggtacgcaccttcccgtccgtccggcagtcctcaggcctctactcgctgagcagcgtggtgagcgtgacctcaagcagccagcccgtcacctgcaacgtggcccacccagccaccaacaccaaagtggacaagaccgttgcgccctcgacatgcagcaagcccatgtgcccaccccctgaactcctggggggaccgtctgtcttcatcttccccccaaaacccaaggacaccctcatgatctcacgcacccccgaggtcacatgcgtggtggtggacgtgagccaggatgaccccgaggtgcagttcacatggtacataaacaacgagcaggtgcgcaccgcccggccgccgctacgggagcagcagttcaacagcacgatccgcgtggtcagcaccctccccatcgcgcaccaggactggctgaggggcaaggagttcaagtgcaaagtccacaacaaggcactcccggcccccatcgagaaaaccatctccaaagccagagggcagcccctggagccgaaggtctacaccatgggccctccccgggaggagctgagcagcaggtcggtcagcctgacctgcatgatcaacggcttctacccttccgacatctcggtggagtgggagaagaacgggaaggcagaggacaactacaagaccacgccggccgtgctggacagcgacggctcctacttcctctacagcaagctctcagtgcccacgagtgagtggcagcggggcgacgtcttcacctgctccgtgatgcacgaggccttgcacaaccactacacgcagaagtccatctcccgctctccgggtaaatga

SEQ ID NO: 73 - DNA, 1329 bp, synthetic construct
  source 1..1329: mol_type = other DNA; note = anti-GAA 376 (clone pEB0613B-4B1-H2) heavy chain coding sequence without leader sequence
caggagcacctggtggagtccgggggaggcctggtcaaccctggaggatccctgacactcacctgcacagcctctggattctccctcaacagcgtcgacatgagctgggtccgccaggctccagggaaggggctggagtggatcggattcagtaatgcttatcataggacatactacgcgagctggtcgaaaagccgatccaccatcaccagaaacaccaacgagaacacggtgactctgaaaatgaccagtctgacagccgcggacacggccacctatttctgtgcgagaggtgttcctggttatgttactaaaagtagtctctggggcccaggcaccctggtcaccgtctcctcagggcaacctaaggctccatcagtcttcccactggccccctgctgcggggacacacccagctccacggtgaccctgggctgcctggtcaaaggctacctcccggagccagtgaccgtgacctggaactcgggcaccctcaccaatggggtacgcaccttcccgtccgtccggcagtcctcaggcctctactcgctgagcagcgtggtgagcgtgacctcaagcagccagcccgtcacctgcaacgtggcccacccagccaccaacaccaaagtggacaagaccgttgcgccctcgacatgcagcaagcccatgtgcccaccccctgaactcctggggggaccgtctgtcttcatcttccccccaaaacccaaggacaccctcatgatctcacgcacccccgaggtcacatgcgtggtggtggacgtgagccaggatgaccccgaggtgcagttcacatggtacataaacaacgagcaggtgcgcaccgcccggccgccgctacgggagcagcagttcaacagcacgatccgcgtggtcagcaccctccccatcgcgcaccaggactggctgaggggcaaggagttcaagtgcaaagtccacaacaaggcactcccggcccccatcgagaaaaccatctccaaagccagagggcagcccctggagccgaaggtctacaccatgggccctccccgggaggagctgagcagcaggtcggtcagcctgacctgcatgatcaacggcttctacccttccgacatctcggtggagtgggagaagaacgggaaggcagaggacaactacaagaccacgccggccgtgctggacagcgacggctcctacttcctctacagcaagctctcagtgcccacgagtgagtggcagcggggcgacgtcttcacctgctccgtgatgcacgaggccttgcacaaccactacacgcagaagtccatctcccgctctccgggtaaatga

SEQ ID NO: 74 - DNA, 414 bp, synthetic construct
  source 1..414: mol_type = other DNA; note = anti-GAA 376 (clone pEB0613B-4B1-H2) variable heavy domain coding sequence with leader sequence
atggagactgggctgcgctggcttctcctggtcgctgtgctcaaaggtgtccagtgtcaggagcacctggtggagtccgggggaggcctggtcaaccctggaggatccctgacactcacctgcacagcctctggattctccctcaacagcgtcgacatgagctgggtccgccaggctccagggaaggggctggagtggatcggattcagtaatgcttatcataggacatactacgcgagctggtcgaaaagccgatccaccatcaccagaaacaccaacgagaacacggtgactctgaaaatgaccagtctgacagccgcggacacggccacctatttctgtgcgagaggtgttcctggttatgttactaaaagtagtctctggggcccaggcaccctggtcaccgtctcctca

SEQ ID NO: 75 - DNA, 357 bp, synthetic construct
  source 1..357: mol_type = other DNA; note = anti-GAA 376 (clone pEB0613B-4B1-H2) variable heavy domain coding sequence with leader sequence
caggagcacctggtggagtccgggggaggcctggtcaaccctggaggatccctgacactcacctgcacagcctctggattctccctcaacagcgtcgacatgagctgggtccgccaggctccagggaaggggctggagtggatcggattcagtaatgcttatcataggacatactacgcgagctggtcgaaaagccgatccaccatcaccagaaacaccaacgagaacacggtgactctgaaaatgaccagtctgacagccgcggacacggccacctatttctgtgcgagaggtgttcctggttatgttactaaaagtagtctctggggcccaggcaccctggtcaccgtctcctca

SEQ ID NO: 76 - protein, 461 aa, synthetic construct
  source 1..461: note = anti-GAA 376 heavy chain amino acid sequence with leader sequence
METGLRWLLLVAVLKGVQCQEHLVESGGGLVNPGGSLTLTCTASGFSLNSVDMSWVRQAPGKGLEWIGFSNAYHRTYYASWSKSRSTITRNTNENTVTLKMTSLTAADTATYFCARGVPGYVTKSSLWGPGTLVTVSSGQPKAPSVFPLAPCCGDTPSSTVTLGCLVKGYLPEPVTVTWNSGTLTNGVRTFPSVRQSSGLYSLSSVVSVTSSSQPVTCNVAHPATNTKVDKTVAPSTCSKPMCPPPELLGGPSVFIFPPKPKDTLMISRTPEVTCVVVDVSQDDPEVQFTWYINNEQVRTARPPLREQQFNSTIRVVSTLPIAHQDWLRGKEFKCKVHNKALPAPIEKTISKARGQPLEPKVYTMGPPREELSSRSVSLTCMINGFYPSDISVEWEKNGKAEDNYKTTPAVLDSDGSYFLYSKLSVPTSEWQRGDVFTCSVMHEALHNHYTQKSISRSPGK

SEQ ID NO: 77 - protein, 442 aa, synthetic construct
  source 1..442: note = anti-GAA 376 heavy chain amino acid sequence without leader sequence
QEHLVESGGGLVNPGGSLTLTCTASGFSLNSVDMSWVRQAPGKGLEWIGFSNAYHRTYYASWSKSRSTITRNTNENTVTLKMTSLTAADTATYFCARGVPGYVTKSSLWGPGTLVTVSSGQPKAPSVFPLAPCCGDTPSSTVTLGCLVKGYLPEPVTVTWNSGTLTNGVRTFPSVRQSSGLYSLSSVVSVTSSSQPVTCNVAHPATNTKVDKTVAPSTCSKPMCPPPELLGGPSVFIFPPKPKDTLMISRTPEVTCVVVDVSQDDPEVQFTWYINNEQVRTARPPLREQQFNSTIRVVSTLPIAHQDWLRGKEFKCKVHNKALPAPIEKTISKARGQPLEPKVYTMGPPREELSSRSVSLTCMINGFYPSDISVEWEKNGKAEDNYKTTPAVLDSDGSYFLYSKLSVPTSEWQRGDVFTCSVMHEALHNHYTQKSISRSPGK

SEQ ID NO: 78 - protein, 138 aa, synthetic construct
  source 1..138: note = anti-GAA 376 variable heavy domain amino acid sequence with leader sequence
METGLRWLLLVAVLKGVQCQEHLVESGGGLVNPGGSLTLTCTASGFSLNSVDMSWVRQAPGKGLEWIGFSNAYHRTYYASWSKSRSTITRNTNENTVTLKMTSLTAADTATYFCARGVPGYVTKSSLWGPGTLVTVSS

SEQ ID NO: 79 - protein, 119 aa, synthetic construct
  source 1..119: note = anti-GAA 376 variable heavy domain amino acid sequence without leader sequence
QEHLVESGGGLVNPGGSLTLTCTASGFSLNSVDMSWVRQAPGKGLEWIGFSNAYHRTYYASWSKSRSTITRNTNENTVTLKMTSLTAADTATYFCARGVPGYVTKSSLWGPGTLVTVSS

SEQ ID NO: 80 - DNA, 717 bp, synthetic construct
  source 1..717: mol_type = other DNA; note = anti-GAA 376 (clone pEB0613B-4B1-K2) light chain coding sequence with leader sequence
atggacacgagggcccccactcagctgctggggctcctgctgctctggctcccaggtgccacatttgccatcgtgatgacccagactccatcttccaagtctgtccctgtgggagacacagtcaccatcaattgccaggccagtcagagtgtttatggtaacaacgaattatcctggtatcagcagaaaccaggacaacctcccaagctcctgatctacaaggcttccactctggcatctggggtcccttcgcggttcaaaggcagtggatctgggacacagttcactctcaccatcagtggcgtggagtgtgacgatgctgccacttactactgtgcaggatatagtagtggtgtgattgatgttagtgctttcggcggggggaccgaggtggtggtcaaaggtgatccagttgcacctactgtcctcatcttcccaccagctgctgatcaggtggcaactggaacagtcaccatcgtgtgtgtggcgaataaatactttcccgatgtcaccgtcacctgggaggtggatggcaccacccaaacaactggcatcgagaacagtaaaacaccgcagaattctgcagattgtacctacaacctcagcagcactctgacactgaccagcacacagtacaacagccacaaagagtacacctgcaaggtgacccagggcacgacctcagtcgtccagagcttcaataggggtgactgttag

SEQ ID NO: 81 - DNA, 648 bp, synthetic construct
  source 1..648: mol_type = other DNA; note = anti-GAA 376 (clone pEB0613B-4B1-K2) light chain coding sequence without leader sequence
atcgtgatgacccagactccatcttccaagtctgtccctgtgggagacacagtcaccatcaattgccaggccagtcagagtgtttatggtaacaacgaattatcctggtatcagcagaaaccaggacaacctcccaagctcctgatctacaaggcttccactctggcatctggggtcccttcgcggttcaaaggcagtggatctgggacacagttcactctcaccatcagtggcgtggagtgtgacgatgctgccacttactactgtgcaggatatagtagtggtgtgattgatgttagtgctttcggcggggggaccgaggtggtggtcaaaggtgatccagttgcacctactgtcctcatcttcccaccagctgctgatcaggtggcaactggaacagtcaccatcgtgtgtgtggcgaataaatactttcccgatgtcaccgtcacctgggaggtggatggcaccacccaaacaactggcatcgagaacagtaaaacaccgcagaattctgcagattgtacctacaacctcagcagcactctgacactgaccagcacacagtacaacagccacaaagagtacacctgcaaggtgacccagggcacgacctcagtcgtccagagcttcaataggggtgactgttag

SEQ ID NO: 82 - DNA, 402 bp, synthetic construct
  source 1..402: mol_type = other DNA; note = anti-GAA 376 (clone pEB0613B-4B1-K2) variable light domain coding sequence with leader sequence
atggacacgagggcccccactcagctgctggggctcctgctgctctggctcccaggtgccacatttgccatcgtgatgacccagactccatcttccaagtctgtccctgtgggagacacagtcaccatcaattgccaggccagtcagagtgtttatggtaacaacgaattatcctggtatcagcagaaaccaggacaacctcccaagctcctgatctacaaggcttccactctggcatctggggtcccttcgcggttcaaaggcagtggatctgggacacagttcactctcaccatcagtggcgtggagtgtgacgatgctgccacttactactgtgcaggatatagtagtggtgtgattgatgttagtgctttcggcggggggaccgaggtggtggtcaaa

SEQ ID NO: 83 - DNA, 333 bp, synthetic construct
  source 1..333: mol_type = other DNA; note = anti-GAA 376 (clone pEB0613B-4B1-K2) variable light domain coding sequence without leader sequence
atcgtgatgacccagactccatcttccaagtctgtccctgtgggagacacagtcaccatcaattgccaggccagtcagagtgtttatggtaacaacgaattatcctggtatcagcagaaaccaggacaacctcccaagctcctgatctacaaggcttccactctggcatctggggtcccttcgcggttcaaaggcagtggatctgggacacagttcactctcaccatcagtggcgtggagtgtgacgatgctgccacttactactgtgcaggatatagtagtggtgtgattgatgttagtgctttcggcggggggaccgaggtggtggtcaaa

SEQ ID NO: 84 - protein, 238 aa, synthetic construct
  source 1..238: note = anti-GAA 376 light chain amino acid sequence with leader sequence
MDTRAPTQLLGLLLLWLPGATFAIVMTQTPSSKSVPVGDTVTINCQASQSVYGNNELSWYQQKPGQPPKLLIYKASTLASGVPSRFKGSGSGTQFTLTISGVECDDAATYYCAGYSSGVIDVSAFGGGTEVVVKGDPVAPTVLIFPPAADQVATGTVTIVCVANKYFPDVTVTWEVDGTTQTTGIENSKTPQNSADCTYNLSSTLTLTSTQYNSHKEYTCKVTQGTTSVVQSFNRGDC

SEQ ID NO: 85 - protein, 215 aa, synthetic construct
  source 1..215: note = anti-GAA 376 light chain amino acid sequence without leader sequence
IVMTQTPSSKSVPVGDTVTINCQASQSVYGNNELSWYQQKPGQPPKLLIYKASTLASGVPSRFKGSGSGTQFTLTISGVECDDAATYYCAGYSSGVIDVSAFGGGTEVVVKGDPVAPTVLIFPPAADQVATGTVTIVCVANKYFPDVTVTWEVDGTTQTTGIENSKTPQNSADCTYNLSSTLTLTSTQYNSHKEYTCKVTQGTTSVVQSFNRGDC

SEQ ID NO: 86 - protein, 134 aa, synthetic construct
  source 1..134: note = anti-GAA 376 variable light domain amino acid sequence with leader sequence
MDTRAPTQLLGLLLLWLPGATFAIVMTQTPSSKSVPVGDTVTINCQASQSVYGNNELSWYQQKPGQPPKLLIYKASTLASGVPSRFKGSGSGTQFTLTISGVECDDAATYYCAGYSSGVIDVSAFGGGTEVVVK

SEQ ID NO: 87 - protein, 111 aa, synthetic construct
  source 1..111: note = anti-GAA 376 variable light domain amino acid sequence without leader sequence
IVMTQTPSSKSVPVGDTVTINCQASQSVYGNNELSWYQQKPGQPPKLLIYKASTLASGVPSRFKGSGSGTQFTLTISGVECDDAATYYCAGYSSGVIDVSAFGGGTEVVVK